European Patent Specification EP 4 105 325 B1, published October 2, 2024. Title: Novel adenine phosphoribosyltransferase variant and a method for producing IMP using the same. Applicant: CJ CheilJedang Corporation. The sequence listing filed with the application follows.

SEQUENCE LISTING (10 sequences)

SEQ ID NO: 1 - protein, 182 aa, Artificial Sequence
  Apt_VT
MNSKYSNAREAIKDKIRYVQDFPEDGVLFEDLTPVLADADAFSVVIDGLADECEKLGADLIAGLDARGFLLGSAAAYKLGTGVLAVRKAGKLPPPVLHQEYSLEYGSAALEIPADGAVITGTKIALVDDVLATGGTLAGARQLLESAGAEVVGAVVVLEVEGLGGREKFGNLPISVLNATTE

SEQ ID NO: 2 - DNA, 549 bp, Artificial Sequence
  apt_VT
gtgaactcaaagtattccaatgcccgcgaagccatcaaggataaaatccgctatgtacaggattttccagaagacggtgtgctttttgaagacctgactccggtattagctgatgccgatgccttttcggttgtcatcgatggacttgctgatgaatgtgaaaagctgggcgcggatcttatcgcaggtctggatgcacgtggctttttgcttggctcagccgcagcgtacaagctgggcaccggtgtcctagctgtgcgcaaggctggcaagcttcctcctccagtgctgcaccaggagtactcgctggaatacggctccgcggcgttggagattcctgcggatggggcagtgattacaggcaccaagattgcgcttgtcgatgacgtccttgccaccggcggtacccttgccggtgctcgtcagctactggagtctgctggcgcagaagtcgttggtgctgttgtggttttggaagttgaaggtttagggggacgtgaaaaatttggaaatctccctattagtgtgctgaatgccacaactgaataa

SEQ ID NO: 3 - protein, 182 aa, Artificial Sequence
  Apt_WT
MNSKYSNAREAIKDKIRYVQDFPEDGVLFEDLTPVLADADAFSVVIDGLADECEKLGADLIAGLDARGFLLGSAAAYKLGTGVLAVRKAGKLPPPVLHQEYSLEYGSAALEIPADGAVITGAKIALVDDVLATGGTLAGARQLLESAGAEVVGAVVVLEVEGLGGREKFGNLPISVLNATTE

SEQ ID NO: 4 - DNA, 549 bp, Artificial Sequence
  apt_WT
gtgaactcaaagtattccaatgcccgcgaagccatcaaggataaaatccgctatgtacaggattttccagaagacggtgtgctttttgaagacctgactccggtattagctgatgccgatgccttttcggttgtcatcgatggacttgctgatgaatgtgaaaagctgggcgcggatcttatcgcaggtctggatgcacgtggctttttgcttggctcagccgcagcgtacaagctgggcaccggtgtcctagctgtgcgcaaggctggcaagcttcctcctccagtgctgcaccaggagtactcgctggaatacggctccgcggcgttggagattcctgcggatggggcagtgattacaggcgccaagattgcgcttgtcgatgacgtccttgccaccggcggtacccttgccggtgctcgtcagctactggagtctgctggcgcagaagtcgttggtgctgttgtggttttggaagttgaaggtttagggggacgtgaaaaatttggaaatctccctattagtgtgctgaatgccacaactgaataa

SEQ ID NO: 5 - DNA, 38 bp, Artificial Sequence
  Primer_1F
gtgaattcgagctcggtacccccaatgcccgcgaagcc

SEQ ID NO: 6 - DNA, 33 bp, Artificial Sequence
  Primer_2R
acaagcgcaatcttggtgcctgtaatcactgcc

SEQ ID NO: 7 - DNA, 33 bp, Artificial Sequence
  Primer_3F
ggcagtgattacaggcaccaagattgcgcttgt

SEQ ID NO: 8 - DNA, 39 bp, Artificial Sequence
  Primer_4R
ggtcgactctagaggatcccccaattccacgtcagcgcg

SEQ ID NO: 9 - DNA, 18 bp, Artificial Sequence
  Primer_5F
ggagacaatccacgaggc

SEQ ID NO: 10 - DNA, 18 bp, Artificial Sequence
  Primer_6R
cccgacttgcgaaatacc